European Patent Application EP 4 461 738 A1, published November 13, 2024. Title: Furin sensors and applications thereof. Applicant: Julius-Maximilians-Universität Würzburg. The sequence listing filed with the application follows.

SEQUENCE LISTING (17 sequences)

SEQ ID NO: 1 - protein, 8 aa, synthetic construct
RRARSVAS

SEQ ID NO: 2 - protein, 8 aa, synthetic construct
SSARSVAS

SEQ ID NO: 3 - protein, 8 aa, synthetic construct
GTAMTAGA

SEQ ID NO: 4 - protein, 8 aa, synthetic construct
GTAMGAGA

SEQ ID NO: 5 - protein, 8 aa, synthetic construct
RTAMTAGA

SEQ ID NO: 6 - protein, 8 aa, synthetic construct
RTAMGAGA

SEQ ID NO: 7 - protein, 8 aa, synthetic construct
RTAMSAGA

SEQ ID NO: 8 - protein, 8 aa, synthetic construct
RTAGSAGA

SEQ ID NO: 9 - protein, 10 aa, synthetic construct
  SITE 1: note = acetylated lysine
  SITE 10: note = glutamate modified with Edans (5-((2-Aminoethyl)amino)naphthalene-1-sulfonic acid)
  SITE 1: note = lysine modified with Dabcyl (4-((4-(Dimethylamino)phenyl)azo)benzoic acid)
KRRARSVASE

SEQ ID NO: 10 - protein, 14 aa, synthetic construct
  SITE 1: note = acetylated glutamate
  SITE 12: note = glutamate modified with Edans (5-((2-Aminoethyl)amino)naphthalene-1-sulfonic acid)
  SITE 3: note = lysine modified with Dabcyl (4-((4-(Dimethylamino)phenyl)azo)benzoic acid)
EGKRTAMTAGAEGE

SEQ ID NO: 11 - protein, 5 aa, synthetic construct
  SITE 1: note = lysine modified with Dabcyl (4-((4-(Dimethylamino)phenyl)azo)benzoic acid)
KRRAR

SEQ ID NO: 12 - protein, 5 aa, synthetic construct
  SITE 5: note = glutamate modified with Edans (5-((2-Aminoethyl)amino)naphthalene-1-sulfonic acid)
SVASE

SEQ ID NO: 13 - protein, 8 aa, unidentified
RERRRKKR

SEQ ID NO: 14 - protein, 6 aa, synthetic construct
GSGSGS

SEQ ID NO: 15 - protein, 10 aa, synthetic construct
  SITE 1: note = lysine modified with Dabcyl (4-((4-(Dimethylamino)phenyl)azo)benzoic acid)
  SITE 10: note = glutamate modified with Edans (5-((2-Aminoethyl)amino)naphthalene-1-sulfonic acid)
KRRARSVASE

SEQ ID NO: 16 - protein, 10 aa, synthetic construct
  SITE 1: note = lysine modified with Dabcyl (4-((4-(Dimethylamino)phenyl)azo)benzoic acid)
  SITE 10: note = glutamate modified with Edans (5-((2-Aminoethyl)amino)naphthalene-1-sulfonic acid)
KRTAMTAGAE

SEQ ID NO: 17 - protein, 8 aa, synthetic construct
  VARIANT 1: note = G or R
  VARIANT 4: note = M or G
  VARIANT 5: note = T or G or S
XTAXXAGA